European Patent Specification EP 3 625 254 B1, published December 13, 2023. Title: Three-dimensional structure-based humanization method. Applicant: F. Hoffmann-La Roche AG. The sequence listing filed with the application follows.

SEQUENCE LISTING (49 sequences)

SEQ ID NO: 1 - protein, 122 aa, Cricetulus migratorius
QIQLQESGPGLVKPSQSLSLTCSVTGFSITTSGYYWTWIRQFPGKKLEWMGYIGYNSKTYYNPSLKSRISITRDTSKNQFLLHLNSVTTEDTATYYCARSLYGGYKDAFDSWGQGTLVTVSS

SEQ ID NO: 2 - protein, 12 aa, Cricetulus migratorius
GFSITTSGYYWT

SEQ ID NO: 3 - protein, 16 aa, Cricetulus migratorius
YIGYNSKTYYNPSLKS

SEQ ID NO: 4 - protein, 12 aa, Cricetulus migratorius
SLYGGYKDAFDS

SEQ ID NO: 5 - protein, 107 aa, Cricetulus migratorius
DVVLTQTPATLSAIPGERVTMTCKASQSIGTSLHWYQHRPNETPRLLIKFASRSITGIPSRFSGSGSGTDFTLGINNLEAEDFAIYYCQQSPGFPPTFGSGTKLEIN

SEQ ID NO: 6 - protein, 11 aa, Cricetulus migratorius
KASQSIGTSLH

SEQ ID NO: 7 - protein, 7 aa, Cricetulus migratorius
FASRSIT

SEQ ID NO: 8 - protein, 9 aa, Cricetulus migratorius
QQSPGFPPT

SEQ ID NO: 9 - protein, 121 aa, Mus musculus
QVQLKESGPGLVAPSQSLSITCTVSGFSLDSYGVHWVRQPPGKGLEWLVVIWSDGTTTYNSALKSRLSITKDNSKSQVFLKMNSLQTDDTAIYYCARDTHYRLYYYAMDYWGQGTSVTVSS

SEQ ID NO: 10 - protein, 37 aa, Mus musculus
TVSGFSLTSYGVHWVRQPPDGSTTYNSALKSRLSISK

SEQ ID NO: 11 - protein, 37 aa, Artificial Sequence
  variant HC-2a
AASGFSLDSYYMSWVRQAPDGTTYYADSVKGRFTISR

SEQ ID NO: 12 - protein, 37 aa, Artificial Sequence; identical to SEQ ID NO: 11
  variant HC-2b

SEQ ID NO: 13 - protein, 37 aa, Artificial Sequence
  variant HC-2c
AASGFSLDSYGMHWVRQAPDGTKYYADSVKGRFTISR

SEQ ID NO: 14 - protein, 37 aa, Artificial Sequence
  variant HC-2d
TVSGFSLDSYYWSWIRQPPDGTTNYNPSLKSRVTISV

SEQ ID NO: 15 - protein, 37 aa, Artificial Sequence
  variant HC-2e
AASGFSLDSYGVHWVRQAPDGTTTYNSALKSRFTISR

SEQ ID NO: 16 - protein, 37 aa, Artificial Sequence
  variant HC-2f
AASGFSLDSYGMHWVRQAPGTNKYYADSVKGRFTISR

SEQ ID NO: 17 - protein, 37 aa, Artificial Sequence
  variant HC-2g
AASGFSLDSYGVHWVRQATDGTTTYNSALKSRFTISR

SEQ ID NO: 18 - protein, 37 aa, Artificial Sequence
  variant HC-2h
AASGFTFSSYGVHWVRQATDGTTTYPGSVKGRFTISR

SEQ ID NO: 19 - protein, 37 aa, Artificial Sequence
  variant HC-2i
AVSGFSLDSYGVHWVRQAPDGTTTYNSALKSRLTISR

SEQ ID NO: 20 - protein, 37 aa, Artificial Sequence
  variant HC-2j
TVSGFSLDSYGVSWIRQPPDGTTNYNPALKSRVTISV

SEQ ID NO: 21 - protein, 37 aa, Artificial Sequence; identical to SEQ ID NO: 19
  variant HC-2k

SEQ ID NO: 22 - protein, 37 aa, Artificial Sequence; identical to SEQ ID NO: 20
  variant HC-2l

SEQ ID NO: 23 - protein, 37 aa, Artificial Sequence
  variant HC-2m
TVSGFSLDSYGMHWVRQAPDGTKSYSTSLKSRLTISK

SEQ ID NO: 24 - protein, 37 aa, Homo sapiens
AASGFTVSSNYMSWVRQAPGGSTYYADSVKGRFTISR

SEQ ID NO: 25 - protein, 37 aa, Homo sapiens; identical to SEQ ID NO: 24

SEQ ID NO: 26 - protein, 37 aa, Homo sapiens
AASGFTFSSYGMHWVRQAPGSNKYYADSVKGRFTISR

SEQ ID NO: 27 - protein, 37 aa, Homo sapiens
TVSGGSISSYYWSWIRQPPSGSTNYNPSLKSRVTISV

SEQ ID NO: 28 - protein, 37 aa, Homo sapiens; identical to SEQ ID NO: 24

SEQ ID NO: 29 - protein, 37 aa, Homo sapiens; identical to SEQ ID NO: 26

SEQ ID NO: 30 - protein, 37 aa, Homo sapiens
AASGFTFSSYDMHWVRQATAGDTYYPGSVKGRFTISR

SEQ ID NO: 31 - protein, 37 aa, Homo sapiens; identical to SEQ ID NO: 30

SEQ ID NO: 32 - protein, 37 aa, Homo sapiens; identical to SEQ ID NO: 24

SEQ ID NO: 33 - protein, 37 aa, Homo sapiens; identical to SEQ ID NO: 27

SEQ ID NO: 34 - protein, 37 aa, Homo sapiens; identical to SEQ ID NO: 24

SEQ ID NO: 35 - protein, 37 aa, Homo sapiens
TVSGGSVSSYYWSWIRQPPSGSTNYNPSLKSRVTISV

SEQ ID NO: 36 - protein, 37 aa, Homo sapiens
TVSGFSLSNMGVSWIRQPPNDEKSYSTSLKSRLTISK

SEQ ID NO: 37 - protein, 40 aa, Artificial Sequence
  variant LC-2a
RSSQSLVHSNGDTYFHWYLQKPGQSPRRLIYKVSNRDSGV

SEQ ID NO: 38 - protein, 40 aa, Artificial Sequence
  variant LC-2b
RSSQSLVHSNGDTYLDWYLQKPGQSPQLLIYKVSNRASGV

SEQ ID NO: 39 - protein, 40 aa, Artificial Sequence
  variant LC-2c
KSSQSLVHSNGDTYLYWYLQKPGQPPQLLIYKVSNRFSGV

SEQ ID NO: 40 - protein, 40 aa, Artificial Sequence
  variant LC-2d
RSSQSLVHSNGDTYFHWYLQKPGQSPQLLIYKVSNRFSGV

SEQ ID NO: 41 - protein, 40 aa, Artificial Sequence; identical to SEQ ID NO: 40
  variant LC-2e

SEQ ID NO: 42 - protein, 40 aa, Artificial Sequence; identical to SEQ ID NO: 40
  variant LC-2f

SEQ ID NO: 43 - protein, 40 aa, Homo sapiens
RSSQSLVYSDGNTYLNWFQQRPGQSPRRLIYKVSNRDSGV

SEQ ID NO: 44 - protein, 40 aa, Homo sapiens
RSSQSLLHSNGYNYLDWYLQKPGQSPQLLIYLGSNRASGV

SEQ ID NO: 45 - protein, 40 aa, Homo sapiens
KSSQSLLHSDGKTYLYWYLQKPGQPPQLLIYEVSNRFSGV

SEQ ID NO: 46 - protein, 40 aa, Homo sapiens; identical to SEQ ID NO: 44

SEQ ID NO: 47 - protein, 40 aa, Homo sapiens; identical to SEQ ID NO: 45

SEQ ID NO: 48 - protein, 40 aa, Homo sapiens; identical to SEQ ID NO: 43

SEQ ID NO: 49 - protein, 112 aa, Mus musculus
DVVMTQTPLSLPVSLGDQASISCRSSQSLVHSNGDTYFHWYLQKPGQSPKLLIYKVSNRFSGVPDRFSGSGSGTDFTLKINRVEAEDLGVYFCSQTTHAPFTFGSGTKLEIK